European Patent Application EP 4 239 063 A1, published September 6, 2023. Title: Reduction of encapsulated host-cell DNA in Adeno-associated vectors by inhibition of apoptotic DNA fragmentation. Applicant: CEVEC Pharmaceuticals GmbH. The sequence listing filed with the application follows.

SEQUENCE LISTING (6 sequences)

SEQ ID NO: 1 - DNA, 25 bp, Artificial Sequence
  SV40 PolyA Primer forward
agcaatagcatcacaaatttcacaa

SEQ ID NO: 2 - DNA, 29 bp, Artificial Sequence
  SV40 PolyA Primer reverse
ccagacatgataagatacattgatgagtt

SEQ ID NO: 3 - DNA, 36 bp, Artificial Sequence
  SV40 PolyA Probe
agcatttttttcactgcattctagttgtggtttgtc

SEQ ID NO: 4 - DNA, 15 bp, Artificial Sequence
  hcDNA Alu Primer forward
gaggcgggcggatca

SEQ ID NO: 5 - DNA, 27 bp, Artificial Sequence
  hcDNA Alu Primer reverse
cccggctaatttttgtatttttagtag

SEQ ID NO: 6 - DNA, 24 bp, Artificial Sequence
  hcDNA Alu Probe
cagcctggccaacatggtgaaacc